European Patent Specification EP 3 597 770 B1, published December 4, 2024. Title: A DNA chip for detecting a caries bacteria. Applicant: GC Corporation. The sequence listing filed with the application follows.

SEQUENCE LISTING (42 sequences)

SEQ ID NO: 1 - DNA, 23 bp, Artificial
  Synthetic DNA
cgtattaccgcggctgctggcac

SEQ ID NO: 2 - DNA, 19 bp, Artificial
  Synthetic DNA
cagtttccgatgcagttcc

SEQ ID NO: 3 - DNA, 17 bp, Artificial
  Synthetic DNA
gccgtgacttgctggtt

SEQ ID NO: 4 - DNA, 17 bp, Artificial
  Synthetic DNA
ctgtcctcttctgcact

SEQ ID NO: 5 - DNA, 17 bp, Artificial
  Synthetic DNA
tttcccagtttccgatg

SEQ ID NO: 6 - DNA, 18 bp, Artificial
  Synthetic DNA
ccgtcactgtgtaagctt

SEQ ID NO: 7 - DNA, 18 bp, Artificial
  Synthetic DNA
ttagccgtccctttctgg

SEQ ID NO: 8 - DNA, 18 bp, Artificial
  Synthetic DNA
cacacgttcttgacttac

SEQ ID NO: 9 - DNA, 30 bp, Artificial
  Synthetic DNA
cgtgcattgtcgtgtaggttcgaccctaat

SEQ ID NO: 10 - DNA, 30 bp, Artificial
  Synthetic DNA
gcagctacgttcatacctacgcaaggcatt

SEQ ID NO: 11 - DNA, 30 bp, Artificial
  Synthetic DNA
gaggagataccgaatcggtcgacgacattt

SEQ ID NO: 12 - DNA, 30 bp, Artificial
  Synthetic DNA
tgttgcgtgaaggtcgtgaacgattggcaa

SEQ ID NO: 13 - DNA, 30 bp, Artificial
  Synthetic DNA
cccctactgagcaaacgttgcactaatgga

SEQ ID NO: 14 - DNA, 30 bp, Artificial
  Synthetic DNA
aacaacgaccgagtgcatagtcacgtacga

SEQ ID NO: 15 - DNA, 30 bp, Artificial
  Synthetic DNA
aggagccctaaggtattggcgagaaaagtc

SEQ ID NO: 16 - DNA, 30 bp, Artificial
  Synthetic DNA
ctgagtatccgcatatcttccgaggttgca

SEQ ID NO: 17 - DNA, 30 bp, Artificial
  Synthetic DNA
acttagctgaccgaaggaccataacgctgt

SEQ ID NO: 18 - DNA, 30 bp, Artificial
  Synthetic DNA
tggaagggatccgtagtcaaccgttgactt

SEQ ID NO: 19 - DNA, 30 bp, Artificial
  Synthetic DNA
cggatcgacatacgacgcctacagaatgtt

SEQ ID NO: 20 - DNA, 30 bp, Artificial
  Synthetic DNA
taaacgtctaggcgagactatgagtgctcc

SEQ ID NO: 21 - DNA, 30 bp, Artificial
  Synthetic DNA
cgtatggatcgatccgacgtaccacattag

SEQ ID NO: 22 - DNA, 30 bp, Artificial
  Synthetic DNA
actgcgtatgatcgacacggctaatcgtag

SEQ ID NO: 23 - DNA, 30 bp, Artificial
  Synthetic DNA
ctattcgaccagcgatatcactacgtaggc

SEQ ID NO: 24 - DNA, 459 bp, Artificial
  Synthetic DNA
gtgagaagcctacacaaacgtaacgtcagggctaagacaaacgctaacggtacaccctagatgggagcttgtagctagatcgctaagtcctaccgacatgtaggcatactcacgaaggcaattccctgaaagcctcgtcttatcccgaacttggcatctgctgatacgtcaggttgaacgcgtacatttacctgtcatgcgtgaatggtaagggtcgtattagggtcgaacctacacgacaatgcacgtcgaagcggttgctaatgcacattggctaaggcccacggaacacgaatcacgtgagatcacttactattcgacggaactactatacgcaccgggacatgcaagtagcgtcccacaagcataaggaactctatactcgccatctacgcagctacaggggatacacgtatgagcggttacgaagtaaagccgagatagagcggtctttagaga

SEQ ID NO: 25 - DNA, 459 bp, Artificial
  Synthetic DNA
gtgagaagcctacacaaacgtaacgtcagggctaagacaaacgctaacggtacaccctagatgggagcttgtagctagatcgctaagtcctaccgacatgtaggcatactcacgaaggcaattccctgaaagcctcgtcttatcccgaacttggcatctgctgatacgtcaggttgaacgcgtacatttacctgtcatgcgtggtagccgattgaactaatgccttgcgtaggtatgaacgtagctgctagtcgaggccttgtatgcacattggctaaggcccacggaacacgaatcacgtgagatcacttactattcgacggaactactatacgcaccgggacatgcaagtagcgtcccacaagcataaggaactctatactcgccatctacgcagctacaggggatacacgtatgagcggttacgaagtaaagccgagatagagcggtctttagaga

SEQ ID NO: 26 - DNA, 459 bp, Artificial
  Synthetic DNA
gtgagaagcctacacaaacgtaacgtcagggctaagacaaacgctaacggtacaccctagatgggagcttgtagctagatcgctaagtcctaccgacatgtaggcatactcacgaaggcaattccctgaaagcctcgtcttatcccgaacttggcatctgctgatacgtcaggttgaacgcgtacatttacctgtcatgcgtgtcctcgatacatacgaaatgtcgtcgaccgattcggtatctcctctggcaccgaagacaaatgcacattggctaaggcccacggaacacgaatcacgtgagatcacttactattcgacggaactactatacgcaccgggacatgcaagtagcgtcccacaagcataaggaactctatactcgccatctacgcagctacaggggatacacgtatgagcggttacgaagtaaagccgagatagagcggtctttagaga

SEQ ID NO: 27 - DNA, 459 bp, Artificial
  Synthetic DNA
gtgagaagcctacacaaacgtaacgtcagggctaagacaaacgctaacggtacaccctagatgggagcttgtagctagatcgctaagtcctaccgacatgtaggcatactcacgaaggcaattccctgaaagcctcgtcttatcccgaacttggcatctgctgatacgtcaggttgaacgcgtacatttacctgtcatgcgtgtgctacgctttacgcttgccaatcgttcacgaccttcacgcaacacttgatcgaaccgaaatgcacattggctaaggcccacggaacacgaatcacgtgagatcacttactattcgacggaactactatacgcaccgggacatgcaagtagcgtcccacaagcataaggaactctatactcgccatctacgcagctacaggggatacacgtatgagcggttacgaagtaaagccgagatagagcggtctttagaga

SEQ ID NO: 28 - DNA, 459 bp, Artificial
  Synthetic DNA
gtgagaagcctacacaaacgtaacgtcagggctaagacaaacgctaacggtacaccctagatgggagcttgtagctagatcgctaagtcctaccgacatgtaggcatactcacgaaggcaattccctgaaagcctcgtcttatcccgaacttggcatctgctgatacgtcaggttgaacgcgtacatttacctgtcatgcgtgacaacagacggtacgtccattagtgcaacgtttgctcagtagggggtctaagcgtcacttatgcacattggctaaggcccacggaacacgaatcacgtgagatcacttactattcgacggaactactatacgcaccgggacatgcaagtagcgtcccacaagcataaggaactctatactcgccatctacgcagctacaggggatacacgtatgagcggttacgaagtaaagccgagatagagcggtctttagaga

SEQ ID NO: 29 - DNA, 459 bp, Artificial
  Synthetic DNA
gtgagaagcctacacaaacgtaacgtcagggctaagacaaacgctaacggtacaccctagatgggagcttgtagctagatcgctaagtcctaccgacatgtaggcatactcacgaaggcaattccctgaaagcctcgtcttatcccgaacttggcatctgctgatacgtcaggttgaacgcgtacatttacctgtcatgcgtgggagcagttttcttctcgtacgtgactatgcactcggtcgttgttggaataccggtcgtaatgcacattggctaaggcccacggaacacgaatcacgtgagatcacttactattcgacggaactactatacgcaccgggacatgcaagtagcgtcccacaagcataaggaactctatactcgccatctacgcagctacaggggatacacgtatgagcggttacgaagtaaagccgagatagagcggtctttagaga

SEQ ID NO: 30 - DNA, 459 bp, Artificial
  Synthetic DNA
gtgagaagcctacacaaacgtaacgtcagggctaagacaaacgctaacggtacaccctagatgggagcttgtagctagatcgctaagtcctaccgacatgtaggcatactcacgaaggcaattccctgaaagcctcgtcttatcccgaacttggcatctgctgatacgtcaggttgaacgcgtacatttacctgtcatgcgtgaacgcaatacggtgggacttttctcgccaataccttagggctcctgtgtacctaagcgaaatgcacattggctaaggcccacggaacacgaatcacgtgagatcacttactattcgacggaactactatacgcaccgggacatgcaagtagcgtcccacaagcataaggaactctatactcgccatctacgcagctacaggggatacacgtatgagcggttacgaagtaaagccgagatagagcggtctttagaga

SEQ ID NO: 31 - DNA, 459 bp, Artificial
  Synthetic DNA
gtgagaagcctacacaaacgtaacgtcagggctaagacaaacgctaacggtacaccctagatgggagcttgtagctagatcgctaagtcctaccgacatgtaggcatactcacgaaggcaattccctgaaagcctcgtcttatcccgaacttggcatctgctgatacgtcaggttgaacgcgtacatttacctgtcatgcgtgggatgacggataagttgcaacctcggaagatatgcggatactcagacgtgatatgcgcagatgcacattggctaaggcccacggaacacgaatcacgtgagatcacttactattcgacggaactactatacgcaccgggacatgcaagtagcgtcccacaagcataaggaactctatactcgccatctacgcagctacaggggatacacgtatgagcggttacgaagtaaagccgagatagagcggtctttagaga

SEQ ID NO: 32 - DNA, 459 bp, Artificial
  Synthetic DNA
gtgagaagcctacacaaacgtaacgtcagggctaagacaaacgctaacggtacaccctagatgggagcttgtagctagatcgctaagtcctaccgacatgtaggcatactcacgaaggcaattccctgaaagcctcgtcttatcccgaacttggcatctgctgatacgtcaggttgaacgcgtacatttacctgtcatgcgtgggtgtacatcggatgacagcgttatggtccttcggtcagctaagtaagtccgttttccacatgcacattggctaaggcccacggaacacgaatcacgtgagatcacttactattcgacggaactactatacgcaccgggacatgcaagtagcgtcccacaagcataaggaactctatactcgccatctacgcagctacaggggatacacgtatgagcggttacgaagtaaagccgagatagagcggtctttagaga

SEQ ID NO: 33 - DNA, 459 bp, Artificial
  Synthetic DNA
gtgagaagcctacacaaacgtaacgtcagggctaagacaaacgctaacggtacaccctagatgggagcttgtagctagatcgctaagtcctaccgacatgtaggcatactcacgaaggcaattccctgaaagcctcgtcttatcccgaacttggcatctgctgatacgtcaggttgaacgcgtacatttacctgtcatgcgtgttcagtcaaccggagaagtcaacggttgactacggatcccttccatgtagagctctcacaatgcacattggctaaggcccacggaacacgaatcacgtgagatcacttactattcgacggaactactatacgcaccgggacatgcaagtagcgtcccacaagcataaggaactctatactcgccatctacgcagctacaggggatacacgtatgagcggttacgaagtaaagccgagatagagcggtctttagaga

SEQ ID NO: 34 - DNA, 459 bp, Artificial
  Synthetic DNA
gtgagaagcctacacaaacgtaacgtcagggctaagacaaacgctaacggtacaccctagatgggagcttgtagctagatcgctaagtcctaccgacatgtaggcatactcacgaaggcaattccctgaaagcctcgtcttatcccgaacttggcatctgctgatacgtcaggttgaacgcgtacatttacctgtcatgcgtggcgattgtcgcgttaaacattctgtaggcgtcgtatgtcgatccgggacttcgcttcataatgcacattggctaaggcccacggaacacgaatcacgtgagatcacttactattcgacggaactactatacgcaccgggacatgcaagtagcgtcccacaagcataaggaactctatactcgccatctacgcagctacaggggatacacgtatgagcggttacgaagtaaagccgagatagagcggtctttagaga

SEQ ID NO: 35 - DNA, 459 bp, Artificial
  Synthetic DNA
gtgagaagcctacacaaacgtaacgtcagggctaagacaaacgctaacggtacaccctagatgggagcttgtagctagatcgctaagtcctaccgacatgtaggcatactcacgaaggcaattccctgaaagcctcgtcttatcccgaacttggcatctgctgatacgtcaggttgaacgcgtacatttacctgtcatgcgtgtcgtgtgtcgtgagaggagcactcatagtctcgcctagacgtttatgacgagatatcacgatgcacattggctaaggcccacggaacacgaatcacgtgagatcacttactattcgacggaactactatacgcaccgggacatgcaagtagcgtcccacaagcataaggaactctatactcgccatctacgcagctacaggggatacacgtatgagcggttacgaagtaaagccgagatagagcggtctttagaga

SEQ ID NO: 36 - DNA, 459 bp, Artificial
  Synthetic DNA
gtgagaagcctacacaaacgtaacgtcagggctaagacaaacgctaacggtacaccctagatgggagcttgtagctagatcgctaagtcctaccgacatgtaggcatactcacgaaggcaattccctgaaagcctcgtcttatcccgaacttggcatctgctgatacgtcaggttgaacgcgtacatttacctgtcatgcgtggtagcgtgtaacgcactaatgtggtacgtcggatcgatccatacgcaactttgtaccgagatgcacattggctaaggcccacggaacacgaatcacgtgagatcacttactattcgacggaactactatacgcaccgggacatgcaagtagcgtcccacaagcataaggaactctatactcgccatctacgcagctacaggggatacacgtatgagcggttacgaagtaaagccgagatagagcggtctttagaga

SEQ ID NO: 37 - DNA, 459 bp, Artificial
  Synthetic DNA
gtgagaagcctacacaaacgtaacgtcagggctaagacaaacgctaacggtacaccctagatgggagcttgtagctagatcgctaagtcctaccgacatgtaggcatactcacgaaggcaattccctgaaagcctcgtcttatcccgaacttggcatctgctgatacgtcaggttgaacgcgtacatttacctgtcatgcgtgagcaaccatcttgagctacgattagccgtgtcgatcatacgcagtccgaggcattactgaatgcacattggctaaggcccacggaacacgaatcacgtgagatcacttactattcgacggaactactatacgcaccgggacatgcaagtagcgtcccacaagcataaggaactctatactcgccatctacgcagctacaggggatacacgtatgagcggttacgaagtaaagccgagatagagcggtctttagaga

SEQ ID NO: 38 - DNA, 459 bp, Artificial
  Synthetic DNA
gtgagaagcctacacaaacgtaacgtcagggctaagacaaacgctaacggtacaccctagatgggagcttgtagctagatcgctaagtcctaccgacatgtaggcatactcacgaaggcaattccctgaaagcctcgtcttatcccgaacttggcatctgctgatacgtcaggttgaacgcgtacatttacctgtcatgcgtgggccttctccgaatagcctacgtagtgatatcgctggtcgaataggcggattgctcataaatgcacattggctaaggcccacggaacacgaatcacgtgagatcacttactattcgacggaactactatacgcaccgggacatgcaagtagcgtcccacaagcataaggaactctatactcgccatctacgcagctacaggggatacacgtatgagcggttacgaagtaaagccgagatagagcggtctttagaga

SEQ ID NO: 39 - DNA, 25 bp, Artificial
  Synthetic DNA
gagaagcctacacaaacgtaacgtc

SEQ ID NO: 40 - DNA, 23 bp, Artificial
  Synthetic DNA
ctctaaagaccgctctatctcgg

SEQ ID NO: 41 - DNA, 15 bp, Artificial
  Synthetic DNA
tacgggaggcagcag

SEQ ID NO: 42 - DNA, 19 bp, Artificial
  Synthetic DNA
crgggtatctaatccygtt